European Patent Application EP 4 219 527 A2, published August 2, 2023. Title: ADENOVIRUSES AND METHODS FOR USING ADENOVIRUSES. Applicant: MAYO FOUNDATION FOR MEDICAL EDUCATION AND RESEARCH. Application US 62/770,631, filed November 21, 2018. The sequence listing filed with the application follows.

SEQUENCE LISTING (65 sequences)

SEQ ID NO: 1 - protein, 12 aa, synthetic construct
  REGION 1..12: note = targeting polypeptide
TARGEHKEEELI

SEQ ID NO: 2 - protein, 12 aa, synthetic construct
  REGION 1..12: note = targeting polypeptide
LRQTGAASAVWG

SEQ ID NO: 3 - protein, 12 aa, synthetic construct
  REGION 1..12: note = targeting polypeptide
ARRADTQWRGLE

SEQ ID NO: 4 - protein, 19 aa, synthetic construct
  REGION 1..19: note = targeting polypeptide
GTWLNPGFPPQSCGYATVT

SEQ ID NO: 5 - protein, 9 aa, synthetic construct
  REGION 1..9: note = targeting polypeptide
CDCRGDCFC

SEQ ID NO: 6 - protein, 10 aa, synthetic construct
  REGION 1..10: note = targeting polypeptide
NMSLDVNRKA

SEQ ID NO: 7 - protein, 12 aa, synthetic construct
  REGION 1..12: note = targeting polypeptide
ISLSSHRATWVV

SEQ ID NO: 8 - protein, 20 aa, synthetic construct
  REGION 1..20: note = targeting polypeptide
WTMGLDQLRDSSWAHGGFSA

SEQ ID NO: 9 - protein, 20 aa, synthetic construct
  REGION 1..20: note = targeting polypeptide
WTMGLDQLRGDSSWAHGGFS

SEQ ID NO: 10 - protein, 20 aa, synthetic construct
  REGION 1..20: note = targeting polypeptide
RSVSGTEWVPMNEQHRGAIW

SEQ ID NO: 11 - protein, 20 aa, synthetic construct
  REGION 1..20: note = targeting polypeptide
TELRTHTSKELTIRTAASSD

SEQ ID NO: 12 - protein, 20 aa, synthetic construct
  REGION 1..20: note = targeting polypeptide
DRAIGWQDKLYKLPLGSIHN

SEQ ID NO: 13 - protein, 20 aa, synthetic construct
  REGION 1..20: note = targeting polypeptide
MGSWEKAALWNRVSASSGGA

SEQ ID NO: 14 - protein, 20 aa, synthetic construct
  REGION 1..20: note = targeting polypeptide
MAMGGKPERPADSDNVQVRG

SEQ ID NO: 15 - protein, 20 aa, synthetic construct
  REGION 1..20: note = targeting polypeptide
MASRGDAGEGSTQSNTNVPS

SEQ ID NO: 16 - protein, 20 aa, synthetic construct
  REGION 1..20: note = targeting polypeptide
GPEDTSRAPENQQKTFHRRW

SEQ ID NO: 17 - protein, 20 aa, synthetic construct
  REGION 1..20: note = targeting polypeptide
MGREDVGEQKLISEEDLGGS

SEQ ID NO: 18 - protein, 11 aa, synthetic construct
  REGION 1..11: note = targeting polypeptide
ACDCRGDCFCG

SEQ ID NO: 19 - protein, 12 aa, synthetic construct
  REGION 1..12: note = targeting polypeptide
ACDCREDVCFCG

SEQ ID NO: 20 - protein, 20 aa, synthetic construct
  REGION 1..20: note = targeting polypeptide
GQIPITEPELCCVPWTEAFY

SEQ ID NO: 21 - protein, 20 aa, synthetic construct
  REGION 1..20: note = targeting polypeptide
PQPPNSTAHPNPHKAPPNTT

SEQ ID NO: 22 - protein, 20 aa, synthetic construct
  REGION 1..20: note = targeting polypeptide
VRWFPGGEWGVTHPESLPPP

SEQ ID NO: 23 - protein, 19 aa, synthetic construct
  REGION 1..19: note = targeting polypeptide
KKKKKKKKKKKKKKKKKKK

SEQ ID NO: 24 - protein, 14 aa, synthetic construct
  REGION 1..14: note = targeting polypeptide
GLNDIFEAQKIEWH

SEQ ID NO: 25 - protein, 23 aa, synthetic construct
  REGION 1..23: note = targeting polypeptide
CAAARWKKAFIAVSAANRFKKIS

SEQ ID NO: 26 - protein, 14 aa, synthetic construct
  REGION 1..14: note = targeting polypeptide
EDPGFFNVEIPEFP

SEQ ID NO: 27 - protein, 20 aa, synthetic construct
  REGION 1..20: note = targeting polypeptide
GGHGRVLWPDGWFSLVGISP

SEQ ID NO: 28 - protein, 21 aa, synthetic construct
  REGION 1..21: note = targeting polypeptide
MARTVTANVPGMGEGMVVVPC

SEQ ID NO: 29 - protein, 20 aa, synthetic construct
  REGION 1..20: note = targeting polypeptide
GVSKRGLQCHDFISCSGVPW

SEQ ID NO: 30 - protein, 20 aa, synthetic construct
  REGION 1..20: note = targeting polypeptide
NQSIPKVAGDSKVFCWWCAL

SEQ ID NO: 31 - protein, 20 aa, synthetic construct
  REGION 1..20: note = targeting polypeptide
QSTPPTKHLTIPRHLRNTLI

SEQ ID NO: 32 - protein, 20 aa, synthetic construct
  REGION 1..20: note = targeting polypeptide
DMSFQLVTPFLKALPTGWRG

SEQ ID NO: 33 - protein, 20 aa, synthetic construct
  REGION 1..20: note = targeting polypeptide
GGHGRVLWPDGWFSLVGISP

SEQ ID NO: 34 - protein, 8 aa, synthetic construct
  REGION 1..8: note = targeting polypeptide
FSLVGISP

SEQ ID NO: 35 - protein, 20 aa, synthetic construct
  REGION 1..20: note = targeting polypeptide
QIMMGPSLGYYMPSESIFAY

SEQ ID NO: 36 - protein, 20 aa, synthetic construct
  REGION 1..20: note = targeting polypeptide
ISWDIWRWWYTSEDRDAGSA

SEQ ID NO: 37 - protein, 20 aa, synthetic construct
  REGION 1..20: note = targeting polypeptide
VWGMTTSDHQRKTERLDSPE

SEQ ID NO: 38 - protein, 20 aa, synthetic construct
  REGION 1..20: note = targeting polypeptide
MTSAQTSEKLKAETDRHTAE

SEQ ID NO: 39 - protein, 19 aa, synthetic construct
  REGION 1..19: note = targeting polypeptide
MGSRSAVGDFESAEGSRRP

SEQ ID NO: 40 - protein, 20 aa, synthetic construct
  REGION 1..20: note = targeting polypeptide
MGRTVQSGDGTPAQTQPSVN

SEQ ID NO: 41 - protein, 20 aa, synthetic construct
  REGION 1..20: note = targeting polypeptide
MARTVTANVPGMGEGMVVVP

SEQ ID NO: 42 - protein, 132 aa, synthetic construct
  REGION 1..132: note = Adenovirus E1A N-terminus polypeptide
MRHIICHGGVITEEMAASLLDQLIEEVLADNLPPPSHFEPPTLHELYDLDVTAPEDPNEEAVSQIFPESVMLAVQEGIDLFTFPPAPGSPEPPHLSRQPEQPEQRALGPVSMPNLVPEVIDLTCHEAGFPPS

SEQ ID NO: 43 - protein, 112 aa, synthetic construct
  REGION 1..112: note = E1A N-terminus polypeptide
MRHIEEVLADNLPPPSHFEPPTLHELYDLDVTAPEDPNEEAVSQIFPESVMLAVQEGIDLFTFPPAPGSPEPPHLSRQPEQPEQRALGPVSMPNLVPEVIDLTCHEAGFPPS

SEQ ID NO: 44 - protein, 119 aa, synthetic construct
  REGION 1..119: note = E1A N-terminus polypeptide
MRHIICHGGVITEEMAASLLDQLIEEVLADNLPPPSHFEPPTLHELYDLDVTAPEDPNEEAVSQIFPESVMLAVQEGIDLFTFPPAPGSPEPPHLSRQPEQPEQRALGPVCHEAGFPPS

SEQ ID NO: 45 - protein, 99 aa, synthetic construct
  REGION 1..99: note = E1A N-terminus polypeptide
MRHIEEVLADNLPPPSHFEPPTLHELYDLDVTAPEDPNEEAVSQIFPESVMLAVQEGIDLFTFPPAPGSPEPPHLSRQPEQPEQRALGPVCHEAGFPPS

SEQ ID NO: 46 - protein, 5 aa, synthetic construct
  REGION 1..5: note = Cell Binding Peptide
REDVY

SEQ ID NO: 47 - protein, 12 aa, synthetic construct
  REGION 1..12: note = Breast Cancer Binding Peptide
ISLSSHRATWVV

SEQ ID NO: 48 - protein, 1608 aa, synthetic construct
  REGION 1..1608: note = Probasin-E1 nucleic acid
TCGAGCGACGGTATCGATAAGCTTGGAGCTTATGATAGCATCTTGTTCTTAGTCTTTTTCTTAATAGGGACATAAAGCCCACAAATAAAAATATGCCTGAAGAATGGGACAGGCATTGGGCATTGTCCATGCCTAGTAAAGTACTCCAAGAACCTATTTGTATACTAGATGACACAATGTTCTAGCCAAGCTTGGTAGTCATCATGTTTAAACATCTACCATTCCAGTTAAGAAAATATGATAGCATCTTGTTCTTAGTCTTTTTCTTAATAGGGACATAAAGCCCACAAATAAAAATATGCCTGAAGAATGGGACAGGCATTGGGCATTGTCCATGCCTAGTAAAGTACTCCAAGAACCTATTTGTATACTAGATGACACAATGTCAATGTCTGTGTACAACTGCCAACTGGGATGCAAGACACTGCCCATGCCAATCATCCTGAAAAGCAGCTATAAAAAGCAGGAAGCTACTCTGCACCTTGTCAGTGAGGTCCAGATACCTCCCTCGAGCGGCCGCGACGCGCAGTGTATTTATACCCGGTGAGTTCCTCAAGAGGCCACTCTTGAGTGCCAGCGAGTAGAGTTTTCTCCTCCGAGCCGCTCCGACACCGGGACTGAAAATGAGACATATTATCTGCCACGGAGGTGTTATTACCGAAGAAATGGCCGCCAGTCTTTTGGACCAGCTGATCGAAGAGGTACTGGCTGATAATCTTCCACCTCCTAGCCATTTTGAACCACCTACCCTTCACGAACTGTATGATTTAGACGTGACGGCCCCCGAAGATCCCAACGAGGAGGCGGTTTCGCAGATTTTTCCCGAGTCTGTAATGTTGGCGGTGCAGGAAGGGATTGACTTATTCACTTTTCCGCCGGCGCCCGGTTCTCCGGAGCCGCCTCACCTTTCCCGGCAGCCCGAGCAGCCGGAGCAGAGAGCCTTGGGTCCGGTTTCTATGCCAAACCTTGTGCCGGAGGTGATCGATCTTACCTGCCACGAGGCTGGCTTTCCACCCAGTGACGACGAGGATGAAGAGGGTGAGGAGTTTGTGTTAGATTATGTGGAGCACCCCGGGCACGGTTGCAGGTCTTGTCATTATCACCGGAGGAATACGGGGGACCCAGATATTATGTGTTCGCTTTGCTATATGAGGACCTGTGGCATGTTTGTCTACAGTAAGTGAAAATTATGGGCAGTCGGTGATAGAGTGGTGGGTTTGGTGTGGTAATTTTTTTTTAATTTTTACAGTTTTGTGGTTTAAAGAATTTTGTATTGTGATTTTTTAAAAGGTCCTGTGTCTGAACCTGAGCCTGAGCCCGAGCCAGAACCGGAGCCTGCAAGACCTACCCGGCGTCCTAAATTGGTGCCTGCTATCCTGAGACGCCCGACATCACCTGTGTCTAGAGAATGCAATAGTAGTACGGATAGCTGTGACTCCGGTCCTTCTAACACACCTCCTGAGATACACCCGGTGGTCCCGCTGTGCCCCATTAAACCAGTTGCCGTGAGAGTTGGTGGGCGTCGCCAGGCTGTGGAATGTATCGAGGACTTGCTTAACGAGTCTGGGCAACCTTTGGACTTGAGCTGTAAACGCCCCAGGCCATAAG

SEQ ID NO: 49 - protein, 959 aa, synthetic construct
  REGION 1..959: note = Hexon Polypeptide
MATPSMMPQWSYMHISGQDASEYLSPGLVQFARATETYFSLNNKFRNPTVAPTHDVTTDRSQRLTLRFIPVDREDTAYSYKARFTLAVGDNRVLDMASTYFDIRGVLDRGPTFKPYSGTAYNALAPKGAPNSCEWDEDDTQVQVAAEDDQDDDEEEEQLPQQRNGKKTHVYAQAPFAGEAINKNGLQIGTNGAATEGNKEIYADKTYQPEPQIGESQWNEAESSVAGGRVLKKTTPMKPCYGSYARPTNSNGGQGVMVEQNGKLESQVEMQFFSTSVNAMNEANAIQPKLVLYSEDVNMETPDTHLSYKPGKSDDNSKAMLGQQSMPNRPNYIAFRDNFIGLMYYNSTGNMGVLAGQASQLNAVVDLQDRNTELSYQLLLDSIGDRTRYFSMWNQAVDSYDPDVRIIENHGTEDELPNYCFPLGGIGVTDTYQAIKATNGNGGATTWAQDNTFAERNEIGVGNNFAMEINLNANLWRNFLYSNIALYLPDKLKYNPTNVEISDNPNTYDYMNKRVVAPGLVDCYINLGARWSLDYMDNVNPFNHHRNAGLRYRSMLLGNGRYVPFHIQVPQKFFAIKNLLLLPGSYTYEWNFRKDVNMVLQSSLGNDLRVDGASIKFDSICLYATFFPMAHNTASTLEAMLRNDTNDQSFNDYLSAANMLYPIPANATNVPISIPSRNWAAFRGWAFTRLKTKETPSLGSGYDPYYTYSGSIPYLDGTFYLNHTFKKVAITFDSSVSWPGNDRLLTPNEFEIKRSVDGEGYNVAQCNMTKDWFLVQMLANYNIGYQGFYIPESYKDRMYSFFRNFQPMSRQVVDDTKYKDYQQVGIIHQHNNSGFVGYLAPTMREGQAYPANVPYPLIGKTAVDSITQKKFLCDRTLWRIPFSSNFMSMGALTDLGQNLLYANSAHALDMTFEVDPMDEPTLLYVLFEVFDVVRVHQPHRGVIETVYLRTPFSAGNATT

SEQ ID NO: 50 - protein, 967 aa, synthetic construct
  REGION 1..967: note = Hexon Polypeptide
MATPSMMPQWSYMHISGQDASEYLSPGLVQFARATETYFSLNNKFRNPTVAPTHDVTTDRSQRLTLRFIPVDREDTAYSYKARFTLAVGDNRVLDMASTYFDIRGVLDRGPTFKPYSGTAYNALAPKGAPNSCEWDEDDTQVQVAAEDDQDDDSSCSSGGTEEEEQLPQQRNGKKTHVYAQAPFAGEAINKNGLQIGTNGAATEGNKEIYADKTYQPEPQIGESQWNEAESSVAGGRVLKKTTPMKPCYGSYARPTNSNGGQGVMVEQNGKLESQVEMQFFSTSVNAMNEANAIQPKLVLYSEDVNMETPDTHLSYKPGKSDDNSKAMLGQQSMPNRPNYIAFRDNFIGLMYYNSTGNMGVLAGQASQLNAVVDLQDRNTELSYQLLLDSIGDRTRYFSMWNQAVDSYDPDVRIIENHGTEDELPNYCFPLGGIGVTDTYQAIKATNGNGGATTWAQDNTFAERNEIGVGNNFAMEINLNANLWRNFLYSNIALYLPDKLKYNPTNVEISDNPNTYDYMNKRVVAPGLVDCYINLGARWSLDYMDNVNPFNHHRNAGLRYRSMLLGNGRYVPFHIQVPQKFFAIKNLLLLPGSYTYEWNFRKDVNMVLQSSLGNDLRVDGASIKFDSICLYATFFPMAHNTASTLEAMLRNDTNDQSFNDYLSAANMLYPIPANATNVPISIPSRNWAAFRGWAFTRLKTKETPSLGSGYDPYYTYSGSIPYLDGTFYLNHTFKKVAITFDSSVSWPGNDRLLTPNEFEIKRSVDGEGYNVAQCNMTKDWFLVQMLANYNIGYQGFYIPESYKDRMYSFFRNFQPMSRQVVDDTKYKDYQQVGIIHQHNNSGFVGYLAPTMREGQAYPANVPYPLIGKTAVDSITQKKFLCDRTLWRIPFSSNFMSMGALTDLGQNLLYANSAHALDMTFEVDPMDEPTLLYVLFEVFDVVRVHQPHRGVIETVYLRTPFSAGNATT

SEQ ID NO: 51 - protein, 955 aa, synthetic construct
  REGION 1..955: note = Hexon Polypeptide
MATPSMMPQWSYMHISGQDASEYLSPGLVQFARATETYFSLNNKFRNPTVAPTHDVTTDRSQRLTLRFIPVDREDTAYSYKARFTLAVGDNRVLDMASTYFDIRGVLDRGPTFKPYSGTAYNALAPKGAPNSCEWDEDDTQVQVAAEDDQDDDEEEEQLPQQRNGKKTHVYAQAPFAGEAINKNGLQIGTNGAATEGNKEIYADKTYQPEPQIGESQWNEAESSVAGGRVLKKTTPMKPCYGSYARPTNSNGGQGVMVEQNGKLESQVEMQFFSTSSCSSGGTPKLVLYSEDVNMETPDTHLSYKPGKSDDNSKAMLGQQSMPNRPNYIAFRDNFIGLMYYNSTGNMGVLAGQASQLNAVVDLQDRNTELSYQLLLDSIGDRTRYFSMWNQAVDSYDPDVRIIENHGTEDELPNYCFPLGGIGVTDTYQAIKATNGNGGATTWAQDNTFAERNEIGVGNNFAMEINLNANLWRNFLYSNIALYLPDKLKYNPTNVEISDNPNTYDYMNKRVVAPGLVDCYINLGARWSLDYMDNVNPFNHHRNAGLRYRSMLLGNGRYVPFHIQVPQKFFAIKNLLLLPGSYTYEWNFRKDVNMVLQSSLGNDLRVDGASIKFDSICLYATFFPMAHNTASTLEAMLRNDTNDQSFNDYLSAANMLYPIPANATNVPISIPSRNWAAFRGWAFTRLKTKETPSLGSGYDPYYTYSGSIPYLDGTFYLNHTFKKVAITFDSSVSWPGNDRLLTPNEFEIKRSVDGEGYNVAQCNMTKDWFLVQMLANYNIGYQGFYIPESYKDRMYSFFRNFQPMSRQVVDDTKYKDYQQVGIIHQHNNSGFVGYLAPTMREGQAYPANVPYPLIGKTAVDSITQKKFLCDRTLWRIPFSSNFMSMGALTDLGQNLLYANSAHALDMTFEVDPMDEPTLLYVLFEVFDVVRVHQPHRGVIETVYLRTPFSAGNATT

SEQ ID NO: 52 - protein, 964 aa, synthetic construct
  REGION 1..964: note = Hexon Polypeptide
MATPSMMPQWSYMHISGQDASEYLSPGLVQFARATETYFSLNNKFRNPTVAPTHDVTTDRSQRLTLRFIPVDREDTAYSYKARFTLAVGDNRVLDMASTYFDIRGVLDRGPTFKPYSGTAYNALAPKGAPNSCEWDEDDTQVQVAAEDDQDDDSSGGTEEEEQLPQQRNGKKTHVYAQAPFAGEAINKNGLQIGTNGAATEGNKEIYADKTYQPEPQIGESQWNEAESSVAGGRVLKKTTPMKPCYGSYARPTNSNGGQGVMVEQNGKLESQVEMQFFSTSVNAMNEANAIQPKLVLYSEDVNMETPDTHLSYKPGKSDDNSKAMLGQQSMPNRPNYIAFRDNFIGLMYYNSTGNMGVLAGQASQLNAVVDLQDRNTELSYQLLLDSIGDRTRYFSMWNQAVDSYDPDVRIIENHGTEDELPNYCFPLGGIGVTDTYQAIKATNGNGGATTWAQDNTFAERNEIGVGNNFAMEINLNANLWRNFLYSNIALYLPDKLKYNPTNVEISDNPNTYDYMNKRVVAPGLVDCYINLGARWSLDYMDNVNPFNHHRNAGLRYRSMLLGNGRYVPFHIQVPQKFFAIKNLLLLPGSYTYEWNFRKDVNMVLQSSLGNDLRVDGASIKFDSICLYATFFPMAHNTASTLEAMLRNDTNDQSFNDYLSAANMLYPIPANATNVPISIPSRNWAAFRGWAFTRLKTKETPSLGSGYDPYYTYSGSIPYLDGTFYLNHTFKKVAITFDSSVSWPGNDRLLTPNEFEIKRSVDGEGYNVAQCNMTKDWFLVQMLANYNIGYQGFYIPESYKDRMYSFFRNFQPMSRQVVDDTKYKDYQQVGIIHQHNNSGFVGYLAPTMREGQAYPANVPYPLIGKTAVDSITQKKFLCDRTLWRIPFSSNFMSMGALTDLGQNLLYANSAHALDMTFEVDPMDEPTLLYVLFEVFDVVRVHQPHRGVIETVYLRTPFSAGNATT

SEQ ID NO: 53 - protein, 952 aa, synthetic construct
  REGION 1..952: note = Hexon Polypeptide
MATPSMMPQWSYMHISGQDASEYLSPGLVQFARATETYFSLNNKFRNPTVAPTHDVTTDRSQRLTLRFIPVDREDTAYSYKARFTLAVGDNRVLDMASTYFDIRGVLDRGPTFKPYSGTAYNALAPKGAPNSCEWDEDDTQVQVAAEDDQDDDEEEEQLPQQRNGKKTHVYAQAPFAGEAINKNGLQIGTNGAATEGNKEIYADKTYQPEPQIGESQWNEAESSVAGGRVLKKTTPMKPCYGSYARPTNSNGGQGVMVEQNGKLESQVEMQFFSTSSGGTPKLVLYSEDVNMETPDTHLSYKPGKSDDNSKAMLGQQSMPNRPNYIAFRDNFIGLMYYNSTGNMGVLAGQASQLNAVVDLQDRNTELSYQLLLDSIGDRTRYFSMWNQAVDSYDPDVRIIENHGTEDELPNYCFPLGGIGVTDTYQAIKATNGNGGATTWAQDNTFAERNEIGVGNNFAMEINLNANLWRNFLYSNIALYLPDKLKYNPTNVEISDNPNTYDYMNKRVVAPGLVDCYINLGARWSLDYMDNVNPFNHHRNAGLRYRSMLLGNGRYVPFHIQVPQKFFAIKNLLLLPGSYTYEWNFRKDVNMVLQSSLGNDLRVDGASIKFDSICLYATFFPMAHNTASTLEAMLRNDTNDQSFNDYLSAANMLYPIPANATNVPISIPSRNWAAFRGWAFTRLKTKETPSLGSGYDPYYTYSGSIPYLDGTFYLNHTFKKVAITFDSSVSWPGNDRLLTPNEFEIKRSVDGEGYNVAQCNMTKDWFLVQMLANYNIGYQGFYIPESYKDRMYSFFRNFQPMSRQVVDDTKYKDYQQVGIIHQHNNSGFVGYLAPTMREGQAYPANVPYPLIGKTAVDSITQKKFLCDRTLWRIPFSSNFMSMGALTDLGQNLLYANSAHALDMTFEVDPMDEPTLLYVLFEVFDVVRVHQPHRGVIETVYLRTPFSAGNATT

SEQ ID NO: 54 - protein, 1033 aa, synthetic construct
  REGION 1..1033: note = Hexon Polypeptide
MATPSMMPQWSYMHISGQDASEYLSPGLVQFARATETYFSLNNKFRNPTVAPTHDVTTDRSQRLTLRFIPVDREDTAYSYKARFTLAVGDNRVLDMASTYFDIRGVLDRGPTFKPYSGTAYNALAPKGAPNSCEWDEDDTQVQVAAEDDQDDDSTGEIPAPLAGTVSKILVKEGDTVKAGQTVLVLEAMKMETEINAPTDGKVEKVLVKERDAVQGGQGLIKIGGGTEEEEQLPQQRNGKKTHVYAQAPFAGEAINKNGLQIGTNGAATEGNKEIYADKTYQPEPQIGESQWNEAESSVAGGRVLKKTTPMKPCYGSYARPTNSNGGQGVMVEQNGKLESQVEMQFFSTSVNAMNEANAIQPKLVLYSEDVNMETPDTHLSYKPGKSDDNSKAMLGQQSMPNRPNYIAFRDNFIGLMYYNSTGNMGVLAGQASQLNAVVDLQDRNTELSYQLLLDSIGDRTRYFSMWNQAVDSYDPDVRIIENHGTEDELPNYCFPLGGIGVTDTYQAIKATNGNGGATTWAQDNTFAERNEIGVGNNFAMEINLNANLWRNFLYSNIALYLPDKLKYNPTNVEISDNPNTYDYMNKRVVAPGLVDCYINLGARWSLDYMDNVNPFNHHRNAGLRYRSMLLGNGRYVPFHIQVPQKFFAIKNLLLLPGSYTYEWNFRKDVNMVLQSSLGNDLRVDGASIKFDSICLYATFFPMAHNTASTLEAMLRNDTNDQSFNDYLSAANMLYPIPANATNVPISIPSRNWAAFRGWAFTRLKTKETPSLGSGYDPYYTYSGSIPYLDGTFYLNHTFKKVAITFDSSVSWPGNDRLLTPNEFEIKRSVDGEGYNVAQCNMTKDWFLVQMLANYNIGYQGFYIPESYKDRMYSFFRNFQPMSRQVVDDTKYKDYQQVGIIHQHNNSGFVGYLAPTMREGQAYPANVPYPLIGKTAVDSITQKKFLCDRTLWRIPFSSNFMSMGALTDLGQNLLYANSAHALDMTFEVDPMDEPTLLYVLFEVFDVVRVHQPHRGVIETVYLRTPFSAGNATT

SEQ ID NO: 55 - protein, 1021 aa, synthetic construct
  REGION 1..1021: note = Hexon Polypeptide
MATPSMMPQWSYMHISGQDASEYLSPGLVQFARATETYFSLNNKFRNPTVAPTHDVTTDRSQRLTLRFIPVDREDTAYSYKARFTLAVGDNRVLDMASTYFDIRGVLDRGPTFKPYSGTAYNALAPKGAPNSCEWDEDDTQVQVAAEDDQDDDEEEEQLPQQRNGKKTHVYAQAPFAGEAINKNGLQIGTNGAATEGNKEIYADKTYQPEPQIGESQWNEAESSVAGGRVLKKTTPMKPCYGSYARPTNSNGGQGVMVEQNGKLESQVEMQFFSTSTGEIPAPLAGTVSKILVKEGDTVKAGQTVLVLEAMKMETEINAPTDGKVEKVLVKERDAVQGGQGLIKIGGGTPKLVLYSEDVNMETPDTHLSYKPGKSDDNSKAMLGQQSMPNRPNYIAFRDNFIGLMYYNSTGNMGVLAGQASQLNAVVDLQDRNTELSYQLLLDSIGDRTRYFSMWNQAVDSYDPDVRIIENHGTEDELPNYCFPLGGIGVTDTYQAIKATNGNGGATTWAQDNTFAERNEIGVGNNFAMEINLNANLWRNFLYSNIALYLPDKLKYNPTNVEISDNPNTYDYMNKRVVAPGLVDCYINLGARWSLDYMDNVNPFNHHRNAGLRYRSMLLGNGRYVPFHIQVPQKFFAIKNLLLLPGSYTYEWNFRKDVNMVLQSSLGNDLRVDGASIKFDSICLYATFFPMAHNTASTLEAMLRNDTNDQSFNDYLSAANMLYPIPANATNVPISIPSRNWAAFRGWAFTRLKTKETPSLGSGYDPYYTYSGSIPYLDGTFYLNHTFKKVAITFDSSVSWPGNDRLLTPNEFEIKRSVDGEGYNVAQCNMTKDWFLVQMLANYNIGYQGFYIPESYKDRMYSFFRNFQPMSRQVVDDTKYKDYQQVGIIHQHNNSGFVGYLAPTMREGQAYPANVPYPLIGKTAVDSITQKKFLCDRTLWRIPFSSNFMSMGALTDLGQNLLYANSAHALDMTFEVDPMDEPTLLYVLFEVFDVVRVHQPHRGVIETVYLRTPFSAGNATT

SEQ ID NO: 56 - protein, 1015 aa, synthetic construct
  REGION 1..1015: note = Hexon Polypeptide
MATPSMMPQWSYMHISGQDASEYLSPGLVQFARATETYFSLNNKFRNPTVAPTHDVTTDRSQRLTLRFIPVDREDTAYSYKARFTLAVGDNRVLDMASTYFDIRGVLDRGPTFKPYSGTAYNALAPKGAPNSCEWDEDDTQVQVAAEDDQDDDEEEEQLPQQRNGKKTHVYAQAPFAGEAINKNGLQIGTNGAATEGNKEIYADKTYQPEPQIGESQWNEAESSVAGGRVLKKTTPMKPCYGSYARPTNSNGGQGVMVEQNGKLESQVEMQFFSTSSSNFTREGNVTYKEEMDKVKNCSFNVTTGIRDKKQKVNALFYRLDITPLDENNNNSSEYRLINSGGTPKLVLYSEDVNMETPDTHLSYKPGKSDDNSKAMLGQQSMPNRPNYIAFRDNFIGLMYYNSTGNMGVLAGQASQLNAVVDLQDRNTELSYQLLLDSIGDRTRYFSMWNQAVDSYDPDVRIIENHGTEDELPNYCFPLGGIGVTDTYQAIKATNGNGGATTWAQDNTFAERNEIGVGNNFAMEINLNANLWRNFLYSNIALYLPDKLKYNPTNVEISDNPNTYDYMNKRVVAPGLVDCYINLGARWSLDYMDNVNPFNHHRNAGLRYRSMLLGNGRYVPFHIQVPQKFFAIKNLLLLPGSYTYEWNFRKDVNMVLQSSLGNDLRVDGASIKFDSICLYATFFPMAHNTASTLEAMLRNDTNDQSFNDYLSAANMLYPIPANATNVPISIPSRNWAAFRGWAFTRLKTKETPSLGSGYDPYYTYSGSIPYLDGTFYLNHTFKKVAITFDSSVSWPGNDRLLTPNEFEIKRSVDGEGYNVAQCNMTKDWFLVQMLANYNIGYQGFYIPESYKDRMYSFFRNFQPMSRQVVDDTKYKDYQQVGIIHQHNNSGFVGYLAPTMREGQAYPANVPYPLIGKTAVDSITQKKFLCDRTLWRIPFSSNFMSMGALTDLGQNLLYANSAHALDMTFEVDPMDEPTLLYVLFEVFDVVRVHQPHRGVIETVYLRTPFSAGNATT

SEQ ID NO: 57 - protein, 987 aa, synthetic construct
  REGION 1..987: note = Hexon Polypeptide
MATPSMMPQWSYMHISGQDASEYLSPGLVQFARATETYFSLNNKFRNPTVAPTHDVTTDRSQRLTLRFIPVDREDTAYSYKARFTLAVGDNRVLDMASTYFDIRGVLDRGPTFKPYSGTAYNALAPKGAPNSCEWDEDDTQVQVAAEDDQDDDEEEEQLPQQRNGKKTHVYAQAPFAGEAINKNGLQIGTNGAATEGNKEIYADKTYQPEPQIGESQWNEAESSVAGGRVLKKTTPMKPCYGSYARPTNSNGGQGVMVEQNGKLESQVEMQFFSTSSQAEPDRAHYNIVTFCCKCDQLLRREVYDFAFRDLSGGTPKLVLYSEDVNMETPDTHLSYKPGKSDDNSKAMLGQQSMPNRPNYIAFRDNFIGLMYYNSTGNMGVLAGQASQLNAVVDLQDRNTELSYQLLLDSIGDRTRYFSMWNQAVDSYDPDVRIIENHGTEDELPNYCFPLGGIGVTDTYQAIKATNGNGGATTWAQDNTFAERNEIGVGNNFAMEINLNANLWRNFLYSNIALYLPDKLKYNPTNVEISDNPNTYDYMNKRVVAPGLVDCYINLGARWSLDYMDNVNPFNHHRNAGLRYRSMLLGNGRYVPFHIQVPQKFFAIKNLLLLPGSYTYEWNFRKDVNMVLQSSLGNDLRVDGASIKFDSICLYATFFPMAHNTASTLEAMLRNDTNDQSFNDYLSAANMLYPIPANATNVPISIPSRNWAAFRGWAFTRLKTKETPSLGSGYDPYYTYSGSIPYLDGTFYLNHTFKKVAITFDSSVSWPGNDRLLTPNEFEIKRSVDGEGYNVAQCNMTKDWFLVQMLANYNIGYQGFYIPESYKDRMYSFFRNFQPMSRQVVDDTKYKDYQQVGIIHQHNNSGFVGYLAPTMREGQAYPANVPYPLIGKTAVDSITQKKFLCDRTLWRIPFSSNFMSMGALTDLGQNLLYANSAHALDMTFEVDPMDEPTLLYVLFEVFDVVRVHQPHRGVIETVYLRTPFSAGNATT

SEQ ID NO: 58 - protein, 959 aa, synthetic construct; identical to SEQ ID NO: 49
  REGION 1..959: note = Hexon Polypeptide

SEQ ID NO: 59 - protein, 962 aa, synthetic construct
  REGION 1..962: note = Hexon Polypeptide
MATPSMMPQWSYMHISGQDASEYLSPGLVQFARATETYFSLNNKFRNPTVAPTHDVTTDRSQRLTLRFIPVDREDTAYSYKARFTLAVGDNRVLDMASTYFDIRGVLDRGPTFKPYSGTAYNALAPKGAPNSCEWEQNETAQVDAQELDEEENEANEAQAREQEQAKKTHVYAQAPLSGEAINKNGLQIGTNGAATEGNKEIYADKTYQPEPQIGESQWNEAESSVAGGRVLKKTTPMKPCYGSYARPTNSNGGQGVMVEQNGKLESQVEMQFFSTSVNAMNEANAIQPKLVLYSEDVNMETPDTHLSYKPGKSDDNSKAMLGQQSMPNRPNYIAFRDNFIGLMYYNSTGNMGVLAGQASQLNAVVDLQDRNTELSYQLLLDSIGDRTRYFSMWNQAVDSYDPDVRIIENHGTEDELPNYCFPLGGIGITDTFQAVKTTAANGDQGNTTWQKDSTFAERNEIGVGNNFAMEINLNANLWRNFLYSNIALYLPDKLKYNPTNVEISDNPNTYDYMNKRVVAPGLVDCYINLGARWSLDYMDNVNPFNHPRHAGLRYRSMLLGNGRYVPFHIQVPQKFFAIKNLLLLPGSYTYEWNFRKDVNMVLQSSLGNDLRVDGASIKFDSICLYATFFPMAHNTASTLEAMLRNDTNDQSFNDYLSAANMLYPIPANATNVPISIPSRNWAAFRGWAFTRLKTKETPSLGSGYDPYYTYSGSIPYLDGTFYLNHTFKKVAITFDSSVSWPGNDRLLTPNEFEIKRSVDGEGYNVAQCNMTKDWFLVQMLANYNIGYQGFYIPESYKDRMYSFFRNFQPMSRQVVDDTKYKDYQQVGIIHQHNNSGFVGYLAPTMREGQAYPANVPYPLIGKTAVDSITQKKFLCDRTLWRIPFSSNFMSMGALTDLGQNLLYANSAHALDMTFEVDPMDEPTLLYVLFEVFDVVRVHQPHRGVIETVYLRTPFSAGNATT

SEQ ID NO: 60 - protein, 528 aa, synthetic construct
  REGION 1..528: note = Fiber Polypeptide
MKRARPSEDTFNPVYPYDTETGPPTVPFLTPPFVSPNGFQESPPGVLSLRLSEPLVTSHGMLALKMGSGLSLDQAGNLTSNTITVSQPLKKTKSNITLETSAPLTVSSGALTMATTSPLVVSDNTLTMQSQAPLTVQDSKLSIATKEPLTVLDGKLALQTSAPLSATDNNALTITASPPLTTANGSLAVTMENPLYNNNGKLGLKIGGPLQVATDSHALTLGTGQGVAVHNNLLHTKVTGAIGFDTSGNMELKTGDGLYVDSAGPNQKLHINLNTTKGLAFDNTAITINAGKGLEFETDSSNGNPIKTKIGSGIQYNTNGAMVAKLGTGLSFDSSGAITMGSINNDRLTLWTTPDPSPNCRIASDKDCKLTLALTKCGSQILGTVSALAVSGNMASINGTLSSVNLVLRFDDNGVLMSNSSLDKQYWNFRNGDSTNGQPYTYAVGFMPNLKAYPKTQSKTAKSNIVSQVYLNGDKSKPLHFTITLNGTDETNQVSKYSISFSWSWNSGQYTNDKFATNSYTFSYIAQE

SEQ ID NO: 61 - protein, 324 aa, synthetic construct
  REGION 1..324: note = Fiber Polypeptide
MKRARPSEDTFNPVYPYDTETGPPTVPFLTPPFVSPNGFQESPPGVLTLKCLTPLTTTGGSLQLKVGGGLTVDDTDGTLQENIRATAPITKNNHSVELSIGNGLETQNNKLCAKLGNGLKFNNGDICIKDSINTLWTGINPPPNCQIVENTNTNDGKLTLVLVKNGGLVNGYVSLVGVSDTVNQMFTQKTANIQLRLYFDSSGNLLTDESDLKIPLKNKSSTATSETVASSKAFMPSTTAYPFNTTTRDSENYIHGICYYMTSYDRSLFPLNISIMLNSRMISSNVAYAIQFEWNLNASESPESNIATLTTSPFFFSYITEDDN

SEQ ID NO: 62 - protein, 534 aa, synthetic construct
  REGION 1..534: note = Fiber Polypeptide
MKRARPSEDTFNPVYPYDTETGPPTVPFLTPPFVSPNGFQESPPGVLSLRLSEPLVTSHGMLALKMGSGLSLDQAGNLTSNTITVSQPLKKTKSNITLETSAPLTVSSGALTMATTSPLVVSDNTLTMQSQAPLTVQDSKLSIATKEPLTVLDGKLALQTSAPLSATDNNALTITASPPLTTANGSLAVTMENPLYNNNGKLGLKIGGPLQVATDSHALTLGTGQGVAVHNNLLHTKVTGAIGFDTSGNMELKTGDGLYVDSAGPNQKLHINLNTTKGLAFDNTAITINAGKGLEFETDSSNGNPIKTKIGSGIQYNTNGAMVAKLGTGLSFDSSGAITMGSINNDRLTLWTTPDPSPNCRIASDKDCKLTLALTKCGSQILGTVSALAVSGNMASINGTLSSVNLVLRFDDNGVLMSNSSLDKQYWNFRNGDSTNGQPYTYAVGFMPNLKAYPKTQSKTAKSNIVSQVYLNGDKSKPLHFTITLNGTDETNQVSKYSISFSWSWNSGQYTNDKFATNSYTFSYIAQEKKKKKK

SEQ ID NO: 63 - protein, 425 aa, synthetic construct
  REGION 1..425: note = Fiber Polypeptide
MKRARPSEDTFNPVYPYDTETGPPTVPFLTPPFVSPNGFQESPPGVLSLRLSEPLVTKNGEITLKLGEGVDLDSSGKLISNTATKAAAPLSFSNNTISLNMDHPFYTKDGKLSLQVSPPLNILRTSILNTLALGFGSGLGLRGSALAVQLVSPLTFDTDGNIKLTLDRGLHVTTGDAIESNISWAKGLKFEDGAIATNIGNGLEFGSSSTETGVDDAYPIQVKLGSGLSFDSTGAIMAGNKEDDKLTLWTTPDPSPNCQILAENDAKLTLCLTKCGSQILATVSVLVVGSGNLNPITGTVSSAQVFLRFDANGVLLTEHSTLKKYWGYRQGDSIDGTPYTNAVGFMPNLKAYPKSQSSTTKNNIVGQVYMNGDVSKPMLLTITLNGTDDSNSTYSMSFSYTWTNGSYVGATFGANSYTFSYIAQE

SEQ ID NO: 64 - protein, 432 aa, synthetic construct
  REGION 1..432: note = Fiber Polypeptide
MKRARPSEDTFNPVYPYDTETGPPTVPFLTPPFVSPNGFQESPPGVLSLRLSEPLVTKNGEITLKLGEGVDLDSSGKLISNTATKAAAPLSFSNNTISLNMDHPFYTKDGKLSLQVSPPLNILRTSILNTLALGFGSGLGLRGSALAVQLVSPLTFDTDGNIKLTLDRGLHVTTGDAIESNISWAKGLKFEDGAIATNIGNGLEFGSSSTETGVDDAYPIQVKLGSGLSFDSTGAIMAGNKEDDKLTLWTTPDPSPNCQILAENDAKLTLCLTKCGSQILATVSVLVVGSGNLNPITGTVSSAQVFLRFDANGVLLTEHSTLKKYWGYRQGDSIDGTPYTNAVGFMPNLKAYPKSQSSTTKNNIVGQVYMNGDVSKPMLLTITLNGTDDSNSTYSMSFSYTWTNGSYVGATFGANSYTFSYIAQEKKKKKKK

SEQ ID NO: 65 - protein, 441 aa, synthetic construct
  REGION 1..441: note = Fiber Polypeptide
MKRARPSEDTFNPVYPYDTETGPPTVPFLTPPFVSPNGFQESPPGVLSLRLSEPLVTKNGEITLKLGEGVDLDSSGKLISNTATKAAAPLSFSNNTISLNMDHPFYTKDGKLSLQVSPPLNILRTSILNTLALGFGSGLGLRGSALAVQLVSPLTFDTDGNIKLTLDRGLHVTTGDAIESNISWAKGLKFEDGAIATNIGNGLEFGSSSTETGVDDAYPIQVKLGSGLSFDSTGAIMAGNKEDDKLTLWTTPDPSPNCQILAENDAKLTLCLTKCGSQILATVSVLVVGSGNLNPITGTVSSAQVFLRFDANGVLLTEHSTLKKYWGYRQGDSIDGTPYTNAVGFMPNLKAYPKSQSSTTKNNIVGQVYMNGDVSKPMLLTITLNGTDDSGGSSGKKKKKKKASGGSSTYSMSFSYTWTNGSYVGATFGANSYTFSYIAQE